European Patent Application EP 4 119 162 A1, published January 18, 2023. Title: PVRIG BINDING PROTEIN AND ITS MEDICAL USES. Applicant: Jiangsu Hengrui Medicine Co., Ltd. Shanghai Shengdi Pharmaceutical Co., Ltd. The sequence listing filed with the application follows.

SEQUENCE LISTING (153 sequences)

SEQ ID NO: 1 - protein, 137 aa, Artificial sequence
  his1PVRIG (cyno-PVRIG-his)
TPEVWVQVQMEATELSSFTVHCGFLGPGSISLVTVSWGGPDGAGGTKLAVLHPELGTRQWAPARQARWETQSSISLALEDSGASSPFANTTFCCKFASFPEGSWESCGSLPPSSDPGLSAPPTPVPILRADHHHHHH

SEQ ID NO: 2 - protein, 121 aa, Artificial sequence
  20-HCVR
DVQLVESGGGSVQAGGSLRLSCVASRYTSRTDCMGWFRQAPGKEHEGVAHIDSDGIPRYVDSVKGRFTISQDHAKNTLYLQMNSLKPEDSATYYCVVGFKFDDDYCAPNDWGQGTQVTVSS

SEQ ID NO: 3 - protein, 121 aa, Artificial sequence
  30-HCVR
HVQLVESGGGSVQAGGSLRLSCEASGYSYSGDCMGWFRRAPGKERDEGVATIDNAGRIKYADSVKGRFTISHGNGKYILYLQMNSLKPEDTDMYYCAAGWTFGGNCSPADWGQGTQVTVSS

SEQ ID NO: 4 - protein, 123 aa, Artificial sequence
  38-HCVR
QVQLVESGGGSVQAGGSLRLSCAASPSTYGPSDMAWFRQAPGKQREGVATISAAGRLTYYTDSVRGRFTISRDNAKNTMYLQMNSLKPEDTAMYYCAADFAGGSSLFADYKYWGQGTQVTVSS

SEQ ID NO: 5 - protein, 120 aa, Artificial sequence
  39-HCVR
QVQLVESGGGSVQAGGSLRLSCAASRYTSRTDCMGWFRQAPGKEREGVAHIDSDGIPRYVESVKGRFTISQDHAKNTLYLQMNSLKPEDSATYYCVVGFKFGDYCAPNDWGQGTQVTVSS

SEQ ID NO: 6 - protein, 127 aa, Artificial sequence
  151-HCVR
HVQLVESGGGSVQAGGSLRLSCVASASGFTYRPYCMAWFRQAPGKEREAVAGIDIFGGTTYADSVKGRFTASRDNAGFSLFLQMNDLKPEDTAMYYCAAGDSPDGRCPPLGQGLNYWGQGTQVTVSS

SEQ ID NO: 7 - protein, 5 aa, Artificial sequence
  20 HCDR1
TDCMG

SEQ ID NO: 8 - protein, 16 aa, Artificial sequence
  20 HCDR2
HIDSDGIPRYVDSVKG

SEQ ID NO: 9 - protein, 13 aa, Artificial sequence
  20 HCDR3
GFKFDDDYCAPND

SEQ ID NO: 10 - protein, 5 aa, Artificial sequence
  30 HCDR1
GDCMG

SEQ ID NO: 11 - protein, 16 aa, Artificial sequence
  30 HCDR2
TIDNAGRIKYADSVKG

SEQ ID NO: 12 - protein, 12 aa, Artificial sequence
  30 HCDR3
GWTFGGNCSPAD

SEQ ID NO: 13 - protein, 5 aa, Artificial sequence
  38 HCDR1
PSDMA

SEQ ID NO: 14 - protein, 17 aa, Artificial sequence
  38 HCDR2
TISAAGRLTYYTDSVRG

SEQ ID NO: 15 - protein, 14 aa, Artificial sequence
  38 HCDR3
DFAGGSSLFADYKY

SEQ ID NO: 16 - protein, 5 aa, Artificial sequence
  39 HCDR1
TDCMG

SEQ ID NO: 17 - protein, 16 aa, Artificial sequence
  39 HCDR2
HIDSDGIPRYVESVKG

SEQ ID NO: 18 - protein, 12 aa, Artificial sequence
  39 HCDR3
GFKFGDYCAPND

SEQ ID NO: 19 - protein, 7 aa, Artificial sequence
  151 HCDR1
YRPYCMA

SEQ ID NO: 20 - protein, 16 aa, Artificial sequence
  151 HCDR2
GIDIFGGTTYADSVKG

SEQ ID NO: 21 - protein, 17 aa, Artificial sequence
  151 HCDR3
GDSPDGRCPPLGQGLNY

SEQ ID NO: 22 - protein, 7 aa, Artificial sequence
  20 HCDR1 CHO
RYTSRTD

SEQ ID NO: 23 - protein, 5 aa, Artificial sequence
  20 HCDR2 CHO
DSDGI

SEQ ID NO: 24 - protein, 13 aa, Artificial sequence
  20 HCDR3 CHO
GFKFDDDYCAPND

SEQ ID NO: 25 - protein, 7 aa, Artificial sequence
  30 HCDR1 CHO
GYSYSGD

SEQ ID NO: 26 - protein, 5 aa, Artificial sequence
  30 HCDR2 CHO
DNAGR

SEQ ID NO: 27 - protein, 12 aa, Artificial sequence
  30 HCDR3 CHO
GWTFGGNCSPAD

SEQ ID NO: 28 - protein, 7 aa, Artificial sequence
  38 HCDR1 CHO
PSTYGPS

SEQ ID NO: 29 - protein, 6 aa, Artificial sequence
  38 HCDR2 CHO
SAAGRL

SEQ ID NO: 30 - protein, 14 aa, Artificial sequence
  38 HCDR3 CHO
DFAGGSSLFADYKY

SEQ ID NO: 31 - protein, 7 aa, Artificial sequence
  39 HCDR1 CHO
RYTSRTD

SEQ ID NO: 32 - protein, 5 aa, Artificial sequence
  39 HCDR2 CHO
DSDGI

SEQ ID NO: 33 - protein, 12 aa, Artificial sequence
  39 HCDR3 CHO
GFKFGDYCAPND

SEQ ID NO: 34 - protein, 9 aa, Artificial sequence
  151 HCDR1 CHO
ASGFTYRPY

SEQ ID NO: 35 - protein, 5 aa, Artificial sequence
  151 HCDR2 CHO
DIFGG

SEQ ID NO: 36 - protein, 17 aa, Artificial sequence
  151 HCDR3 CHO
GDSPDGRCPPLGQGLNY

SEQ ID NO: 37 - protein, 8 aa, Artificial sequence
  20 HCDR1 IMGT
RYTSRTDC

SEQ ID NO: 38 - protein, 7 aa, Artificial sequence
  20 HCDR2 IMGT
IDSDGIP

SEQ ID NO: 39 - protein, 15 aa, Artificial sequence
  20 HCDR3 IMGT
VVGFKFDDDYCAPND

SEQ ID NO: 40 - protein, 8 aa, Artificial sequence
  30 HCDR1 IMGT
GYSYSGDC

SEQ ID NO: 41 - protein, 7 aa, Artificial sequence
  30 HCDR2 IMGT
IDNAGRI

SEQ ID NO: 42 - protein, 14 aa, Artificial sequence
  30 HCDR3 IMGT
AAGWTFGGNCSPAD

SEQ ID NO: 43 - protein, 8 aa, Artificial sequence
  38 HCDR1 IMGT
PSTYGPSD

SEQ ID NO: 44 - protein, 8 aa, Artificial sequence
  38 HCDR2 IMGT
ISAAGRLT

SEQ ID NO: 45 - protein, 16 aa, Artificial sequence
  38 HCDR3 IMGT
AADFAGGSSLFADYKY

SEQ ID NO: 46 - protein, 8 aa, Artificial sequence
  39 HCDR1 IMGT
RYTSRTDC

SEQ ID NO: 47 - protein, 7 aa, Artificial sequence
  39 HCDR2 IMGT
IDSDGIP

SEQ ID NO: 48 - protein, 14 aa, Artificial sequence
  39 HCDR3 IMGT
VVGFKFGDYCAPND

SEQ ID NO: 49 - protein, 10 aa, Artificial sequence
  151 HCDR1 IMGT
ASGFTYRPYC

SEQ ID NO: 50 - protein, 7 aa, Artificial sequence
  151 HCDR2 IMGT
IDIFGGT

SEQ ID NO: 51 - protein, 19 aa, Artificial sequence
  151 HCDR3 IMGT
AAGDSPDGRCPPLGQGLNY

SEQ ID NO: 52 - protein, 10 aa, Artificial sequence
  20 HCDR1 ABM
RYTSRTDCMG

SEQ ID NO: 53 - protein, 9 aa, Artificial sequence
  20 HCDR2 ABM
HIDSDGIPR

SEQ ID NO: 54 - protein, 13 aa, Artificial sequence
  20 HCDR3 ABM
GFKFDDDYCAPND

SEQ ID NO: 55 - protein, 10 aa, Artificial sequence
  30 HCDR1 ABM
GYSYSGDCMG

SEQ ID NO: 56 - protein, 9 aa, Artificial sequence
  30 HCDR2 ABM
TIDNAGRIK

SEQ ID NO: 57 - protein, 12 aa, Artificial sequence
  30 HCDR3 ABM
GWTFGGNCSPAD

SEQ ID NO: 58 - protein, 10 aa, Artificial sequence
  38 HCDR1 ABM
PSTYGPSDMA

SEQ ID NO: 59 - protein, 10 aa, Artificial sequence
  38 HCDR2 ABM
TISAAGRLTY

SEQ ID NO: 60 - protein, 14 aa, Artificial sequence
  38 HCDR3 ABM
DFAGGSSLFADYKY

SEQ ID NO: 61 - protein, 10 aa, Artificial sequence
  39 HCDR1 ABM
RYTSRTDCMG

SEQ ID NO: 62 - protein, 9 aa, Artificial sequence
  39 HCDR2 ABM
HIDSDGIPR

SEQ ID NO: 63 - protein, 12 aa, Artificial sequence
  39 HCDR3 ABM
GFKFGDYCAPND

SEQ ID NO: 64 - protein, 12 aa, Artificial sequence
  151 HCDR1 ABM
ASGFTYRPYCMA

SEQ ID NO: 65 - protein, 9 aa, Artificial sequence
  151 HCDR2 ABM
GIDIFGGTT

SEQ ID NO: 66 - protein, 17 aa, Artificial sequence
  151 HCDR3 ABM
GDSPDGRCPPLGQGLNY

SEQ ID NO: 67 - protein, 350 aa, Artificial sequence
  20 HC
DVQLVESGGGSVQAGGSLRLSCVASRYTSRTDCMGWFRQAPGKEHEGVAHIDSDGIPRYVDSVKGRFTISQDHAKNTLYLQMNSLKPEDSATYYCVVGFKFDDDYCAPNDWGQGTQVTVSSESKYGPPCPPCPAPEAAGGPSVFLFPPKPKDTLMISRTPEVTCVVVDVSQEDPEVQFNWYVDGVEVHNAKTKPREEQFNSTYRVVSVLTVLHQDWLNGKEYKCKVSNKGLPSSIEKTISKAKGQPREPQVYTLPPSQEEMTKNQVSLTCLVKGFYPSDIAVEWESNGQPENNYKTTPPVLDSDGSFFLYSRLTVDKSRWQEGNVFSCSVMHEALHNHYTQKSLSLSLGA

SEQ ID NO: 68 - protein, 350 aa, Artificial sequence
  30 HC
HVQLVESGGGSVQAGGSLRLSCEASGYSYSGDCMGWFRRAPGKERDEGVATIDNAGRIKYADSVKGRFTISHGNGKYILYLQMNSLKPEDTDMYYCAAGWTFGGNCSPADWGQGTQVTVSSESKYGPPCPPCPAPEAAGGPSVFLFPPKPKDTLMISRTPEVTCVVVDVSQEDPEVQFNWYVDGVEVHNAKTKPREEQFNSTYRVVSVLTVLHQDWLNGKEYKCKVSNKGLPSSIEKTISKAKGQPREPQVYTLPPSQEEMTKNQVSLTCLVKGFYPSDIAVEWESNGQPENNYKTTPPVLDSDGSFFLYSRLTVDKSRWQEGNVFSCSVMHEALHNHYTQKSLSLSLGA

SEQ ID NO: 69 - protein, 352 aa, Artificial sequence
  38 HC
QVQLVESGGGSVQAGGSLRLSCAASPSTYGPSDMAWFRQAPGKQREGVATISAAGRLTYYTDSVRGRFTISRDNAKNTMYLQMNSLKPEDTAMYYCAADFAGGSSLFADYKYWGQGTQVTVSSESKYGPPCPPCPAPEAAGGPSVFLFPPKPKDTLMISRTPEVTCVVVDVSQEDPEVQFNWYVDGVEVHNAKTKPREEQFNSTYRVVSVLTVLHQDWLNGKEYKCKVSNKGLPSSIEKTISKAKGQPREPQVYTLPPSQEEMTKNQVSLTCLVKGFYPSDIAVEWESNGQPENNYKTTPPVLDSDGSFFLYSRLTVDKSRWQEGNVFSCSVMHEALHNHYTQKSLSLSLGA

SEQ ID NO: 70 - protein, 349 aa, Artificial sequence
  39 HC
QVQLVESGGGSVQAGGSLRLSCAASRYTSRTDCMGWFRQAPGKEREGVAHIDSDGIPRYVESVKGRFTISQDHAKNTLYLQMNSLKPEDSATYYCVVGFKFGDYCAPNDWGQGTQVTVSSESKYGPPCPPCPAPEAAGGPSVFLFPPKPKDTLMISRTPEVTCVVVDVSQEDPEVQFNWYVDGVEVHNAKTKPREEQFNSTYRVVSVLTVLHQDWLNGKEYKCKVSNKGLPSSIEKTISKAKGQPREPQVYTLPPSQEEMTKNQVSLTCLVKGFYPSDIAVEWESNGQPENNYKTTPPVLDSDGSFFLYSRLTVDKSRWQEGNVFSCSVMHEALHNHYTQKSLSLSLGA

SEQ ID NO: 71 - protein, 356 aa, Artificial sequence
  151 HC
HVQLVESGGGSVQAGGSLRLSCVASASGFTYRPYCMAWFRQAPGKEREAVAGIDIFGGTTYADSVKGRFTASRDNAGFSLFLQMNDLKPEDTAMYYCAAGDSPDGRCPPLGQGLNYWGQGTQVTVSSESKYGPPCPPCPAPEAAGGPSVFLFPPKPKDTLMISRTPEVTCVVVDVSQEDPEVQFNWYVDGVEVHNAKTKPREEQFNSTYRVVSVLTVLHQDWLNGKEYKCKVSNKGLPSSIEKTISKAKGQPREPQVYTLPPSQEEMTKNQVSLTCLVKGFYPSDIAVEWESNGQPENNYKTTPPVLDSDGSFFLYSRLTVDKSRWQEGNVFSCSVMHEALHNHYTQKSLSLSLGA

SEQ ID NO: 72 - protein, 449 aa, Artificial sequence
  tab5 HC
EVQLVESGGGVVKPGGSLRLSCAASGFTFGTSSMNWVRQAPGKGLEWVAVISFDGTEIHYADSVKGRFTISRDNSKSTVFLQMNSLRPDDTALYYCAKGSGNIYFYSGMDVWGQGTTVTVSSASTKGPSVFPLAPCSRSTSESTAALGCLVKDYFPEPVTVSWNSGALTSGVHTFPAVLQSSGLYSLSSVVTVPSSSLGTKTYTCNVDHKPSNTKVDKRVESKYGPPCPPCPAPEAAGGPSVFLFPPKPKDTLMISRTPEVTCVVVDVSQEDPEVQFNWYVDGVEVHNAKTKPREEQFNSTYRVVSVLTVLHQDWLNGKEYKCKVSNKGLPSSIEKTISKAKGQPREPQVYTLPPSQEEMTKNQVSLTCLVKGFYPSDIAVEWESNGQPENNYKTTPPVLDSDGSFFLYSRLTVDKSRWQEGNVFSCSVMHEALHNHYTQKSLSLSLGA

SEQ ID NO: 73 - protein, 214 aa, Artificial sequence
  tab5 LC
DIQMTQSPSTLSASVGDRVTITCRAGQSISGWLAWFQQKPGKAPNLLIYETSTLESGVPSRFSGSGSGTEYTLTISSLQPDDFATYYCQQYYSYPLTFGQGTKVEIKRTVAAPSVFIFPPSDEQLKSGTASVVCLLNNFYPREAKVQWKVDNALQSGNSQESVTEQDSKDSTYSLSSTLTLSKADYEKHKVYACEVTHQGLSSPVTKSFNRGEC

SEQ ID NO: 74 - protein, 98 aa, Artificial sequence
  IGHV3-7 *01 HCVR
EVQLVESGGGLVQPGGSLRLSCAASGFTFSSYWMSWVRQAPGKGLEWVANIKQDGSEKYYVDSVKGRFTISRDNAKNSLYLQMNSLRAEDTAVYYCAR

SEQ ID NO: 75 - protein, 121 aa, Artificial sequence
  20H1 HCVR
EVQLVESGGGLVQPGGSLRLSCAASGFTFSTDCMGWFRQAPGKGLEGVAHIDSDGIPRYVDSVKGRFTISRDNAKNSLYLQMNSLRAEDTAVYYCVVGFKFDEDYCAPNDWGQGTMVTVSS

SEQ ID NO: 76 - protein, 121 aa, Artificial sequence
  20H2 HCVR
EVQLVESGGGLVQPGGSLRLSCAASGFTSRTDCMGWFRQAPGKGLEGVAHIDSDGIPRYVDSVKGRFTISRDNAKNSLYLQMNSLRAEDTAVYYCVVGFKFDEDYCAPNDWGQGTMVTVSS

SEQ ID NO: 77 - protein, 121 aa, Artificial sequence
  20H3 HCVR
EVQLVESGGGLVQPGGSLRLSCAASGYTFSTDCMGWFRQAPGKGLEGVAHIDSDGIPRYVDSVKGRFTISQDHAKNSLYLQMNSLRAEDTAVYYCVVGFKFDEDYCAPNDWGQGTMVTVSS

SEQ ID NO: 78 - protein, 121 aa, Artificial sequence
  20H4 HCVR
EVQLVESGGGLVQPGGSLRLSCAASGYTSRTDCMGWFRQAPGKGLEGVAHIDSDGIPRYVDSVKGRFTISQDHAKNSLYLQMNSLRAEDTAVYYCVVGFKFDEDYCAPNDWGQGTMVTVSS

SEQ ID NO: 79 - protein, 121 aa, Artificial sequence
  20H5 HCVR
EVQLVESGGGLVQPGGSLRLSCAASGYTSRTDCMGWFRQAPGKEHEGVAHIDSDGIPRYVDSVKGRFTISQDHAKNSLYLQMNSLRAEDTAVYYCVVGFKFDEDYCAPNDWGQGTMVTVSS

SEQ ID NO: 80 - protein, 120 aa, Artificial sequence
  30H1 HCVR
EVQLVESGGGLVQPGGSLRLSCAASGFTFSGDCMGWFRQAPGKGLEGVATIDNAGRIKYADSVKGRFTISRDNAKNSLYLQMNSLRAEDTAVYYCAAGWTFGGQCSPADWGQGTQVTVSS

SEQ ID NO: 81 - protein, 121 aa, Artificial sequence
  30H2 HCVR
EVQLVESGGGLVQPGGSLRLSCAASGFTFSGDCMGWFRQAPGKGLDEGVATIDNAGRIKYADSVKGRFTISRDNAKNSLYLQMNSLRAEDTAVYYCAAGWTFGGQCSPADWGQGTQVTVSS

SEQ ID NO: 82 - protein, 121 aa, Artificial sequence
  30H3 HCVR
EVQLVESGGGLVQPGGSLRLSCAASGYSYSGDCMGWFRQAPGKGLDEGVATIDNAGRIKYADSVKGRFTISRDNAKNSLYLQMNSLRAEDTAVYYCAAGWTFGGQCSPADWGQGTQVTVSS

SEQ ID NO: 83 - protein, 121 aa, Artificial sequence
  30H4 HCVR
EVQLVESGGGLVQPGGSLRLSCAASGFTFSGDCMGWFRQAPGKGLDEGVATIDNAGRIKYADSVKGRFTISHGNAKYILYLQMNSLRAEDTAVYYCAAGWTFGGQCSPADWGQGTQVTVSS

SEQ ID NO: 84 - protein, 121 aa, Artificial sequence
  30H5 HCVR
EVQLVESGGGLVQPGGSLRLSCAASGYSYSGDCMGWFRQAPGKGLDEGVATIDNAGRIKYADSVKGRFTISHGNAKYILYLQMNSLRAEDTAVYYCAAGWTFGGQCSPADWGQGTQVTVSS

SEQ ID NO: 85 - protein, 98 aa, Artificial sequence
  IGHV3-30 *02
QVQLVESGGGVVQPGGSLRLSCAASGFTFSSYGMHWVRQAPGKGLEWVAFIRYDGSNKYYADSVKGRFTISRDNSKNTLYLQMNSLRAEDTAVYYCAK

SEQ ID NO: 86 - protein, 123 aa, Artificial sequence
  38H2 HCVR
EVQLVESGGGVVQPGGSLRLSCAASGFTFSPSDMAWFRQAPGKGLEGVATISAAGRLTYYTDSVRGRFTISRDNSKNTLYLQMNSLRAEDTAVYYCAADFAGGSSLFADYKYWGQGTMVTVSS

SEQ ID NO: 87 - protein, 123 aa, Artificial sequence
  38H4 HCVR
EVQLVESGGGVVQPGGSLRLSCAASPFTYGPSDMAWFRQAPGKGLEGVATISAAGRLTYYTDSVRGRFTISRDNSKNTLYLQMNSLRAEDTAVYYCAADFAGGSSLFADYKYWGQGTMVTVSS

SEQ ID NO: 88 - protein, 123 aa, Artificial sequence
  38H7 HCVR
EVQLVESGGGVVQPGGSLRLSCAASPSTYGPSDMAWFRQAPGKQREGVATISAAGRLTYYTDSVRGRFTISRDNSKNTMYLQMNSLRAEDTAVYYCAADFAGGSSLFADYKYWGQGTMVTVSS

SEQ ID NO: 89 - protein, 123 aa, Artificial sequence
  38H8 HCVR
EVQLVESGGGVVQPGGSLRLSCAASPSTYGPSDMAWFRQAPGKGLEGVATISAAGRLTYYTDSVRGRFTISRDNSKNTLYLQMNSLRAEDTAVYYCAADFAGGSSLFADYKYWGQGTMVTVSS

SEQ ID NO: 90 - protein, 123 aa, Artificial sequence
  38H9 HCVR
EVQLVESGGGVVQPGGSLRLSCAASPSTYGPSDMAWFRQAPGKGLEGVATISAAGRLTYYTDSVRGRFTISRDNSKNTMYLQMNSLRAEDTAVYYCAADFAGGSSLFADYKYWGQGTMVTVSS

SEQ ID NO: 91 - protein, 120 aa, Artificial sequence
  39H1 HCVR
EVQLVESGGGLVQPGGSLRLSCAASGFTFSTDCMGWFRQAPGKGLEGVAHIDSDGIPRYVESVKGRFTISRDNAKNSLYLQMNSLRAEDTAVYYCVVGFKFGDYCAPNDWGQGTMVTVSS

SEQ ID NO: 92 - protein, 120 aa, Artificial sequence
  39H2 HCVR
EVQLVESGGGLVQPGGSLRLSCAASGFTSRTDCMGWFRQAPGKGLEGVAHIDSDGIPRYVESVKGRFTISRDNAKNSLYLQMNSLRAEDTAVYYCVVGFKFGDYCAPNDWGQGTMVTVSS

SEQ ID NO: 93 - protein, 120 aa, Artificial sequence
  39H3 HCVR
EVQLVESGGGLVQPGGSLRLSCAASGYTFSTDCMGWFRQAPGKGLEGVAHIDSDGIPRYVESVKGRFTISQDHAKNSLYLQMNSLRAEDTAVYYCVVGFKFGDYCAPNDWGQGTMVTVSS

SEQ ID NO: 94 - protein, 120 aa, Artificial sequence
  39H4 HCVR
EVQLVESGGGLVQPGGSLRLSCAASGYTSRTDCMGWFRQAPGKGLEGVAHIDSDGIPRYVESVKGRFTISQDHAKNSLYLQMNSLRAEDTAVYYCVVGFKFGDYCAPNDWGQGTMVTVSS

SEQ ID NO: 95 - protein, 120 aa, Artificial sequence
  39H5 HCVR
EVQLVESGGGLVQPGGSLRLSCAASGYTSRTDCMGWFRQAPGKEREGVAHIDSDGIPRYVESVKGRFTISQDHAKNSLYLQMNSLRAEDTAVYYCVVGFKFGDYCAPNDWGQGTMVTVSS

SEQ ID NO: 96 - protein, 125 aa, Artificial sequence
  151H2 HCVR
EVQLVESGGGLVQPGGSLRLSCAASGFTYRPYCMAWFRQAPGKGLEAVAGIDIFGGTTYADSVKGRFTISRDNAKNSLYLQMNSLRAEDTAVYYCAAGDSPDGRCPPLGQGLNYWGQGTMVTVSS

SEQ ID NO: 97 - protein, 127 aa, Artificial sequence
  151H4 HCVR
EVQLVESGGGLVQPGGSLRLSCVASASGFTYRPYCMAWFRQAPGKGLEAVAGIDIFGGTTYADSVKGRFTISRDNAKNSLYLQMNSLRAEDTAVYYCAAGDSPDGRCPPLGQGLNYWGQGTMVTVSS

SEQ ID NO: 98 - protein, 127 aa, Artificial sequence
  151H7 HCVR
HVQLVESGGGLVQPGGSLRLSCVASASGFTYRPYCMAWFRQAPGKEREAVAGIDIFGGTTYADSVKGRFTASRDNAGFSLYLQMNSLRAEDTAVYYCAAGDSPDGRCPPLGQGLNYWGQGTMVTVSS

SEQ ID NO: 99 - protein, 127 aa, Artificial sequence
  151H8 HCVR
EVQLVESGGGLVQPGGSLRLSCVASASGFTYRPYCMAWFRQAPGKGLEAVAGIDIFGGTTYADSVKGRFTISRDNAGFSLYLQMNSLRAEDTAVYYCAAGDSPDGRCPPLGQGLNYWGQGTMVTVSS

SEQ ID NO: 100 - protein, 127 aa, Artificial sequence
  151H9 HCVR
HVQLVESGGGLVQPGGSLRLSCVASASGFTYRPYCMAWFRQAPGKGLEAVAGIDIFGGTTYADSVKGRFTASRDNAGFSLYLQMNSLRAEDTAVYYCAAGDSPDGRCPPLGQGLNYWGQGTMVTVSS

SEQ ID NO: 101 - protein, 229 aa, Artificial sequence
  Fc region of human IgG4 heavy chain (S228P/F234A/L235A/K447A)
ESKYGPPCPPCPAPEAAGGPSVFLFPPKPKDTLMISRTPEVTCVVVDVSQEDPEVQFNWYVDGVEVHNAKTKPREEQFNSTYRVVSVLTVLHQDWLNGKEYKCKVSNKGLPSSIEKTISKAKGQPREPQVYTLPPSQEEMTKNQVSLTCLVKGFYPSDIAVEWESNGQPENNYKTTPPVLDSDGSFFLYSRLTVDKSRWQEGNVFSCSVMHEALHNHYTQKSLSLSLGA

SEQ ID NO: 102 - protein, 446 aa, Artificial sequence
  1708TIGITHC
EVQLVQSGAEVKKPGASVKVSCKASGYTFTNYWMHWVRQAPGQGLEWMGRIDPDSTGSKYNEKFKTRVTMTRDTSTSTVYMELSSLRSEDTAVYYCAREGAYGYYFDYWGQGTLVTVSSASTKGPSVFPLAPCSRSTSESTAALGCLVKDYFPEPVTVSWNSGALTSGVHTFPAVLQSSGLYSLSSVVTVPSSSLGTKTYTCNVDHKPSNTKVDKRVESKYGPPCPPCPAPEFLGGPSVFLFPPKPKDTLMISRTPEVTCVVVDVSQEDPEVQFNWYVDGVEVHNAKTKPREEQFNSTYRVVSVLTVLHQDWLNGKEYKCKVSNKGLPSSIEKTISKAKGQPREPQVYTLPPSQEEMTKNQVSLTCLVKGFYPSDIAVEWESNGQPENNYKTTPPVLDSDGSFFLYSRLTVDKSRWQEGNVFSCSVMHEALHNHYTQKSLSLSLGK

SEQ ID NO: 103 - protein, 214 aa, Artificial sequence
  1708TIGIT LC
DIQMTQSPSSLSASVGDRVTITCRASENIYSYLAWYQQKPGKSPKLLIYNARTLAEGVPSRFSGSGSGTDFTLTISSLQPEDFATYYCQYHSGSPLPFGGGTKVEIKRTVAAPSVFIFPPSDEQLKSGTASVVCLLNNFYPREAKVQWKVDNALQSGNSQESVTEQDSKDSTYSLSSTLTLSKADYEKHKVYACEVTHQGLSSPVTKSFNRGEC

SEQ ID NO: 104 - protein, 583 aa, Artificial sequence
  1708-151-11511708N
HVQLVESGGGSVQAGGSLRLSCVASASGFTYRPYCMAWFRQAPGKEREAVAGIDIFGGTTYADSVKGRFTASRDNAGFSLFLQMNDLKPEDTAMYYCAAGDSPDGRCPPLGQGLNYWGQGTQVTVSSGGGGSGGGGSEVQLVQSGAEVKKPGASVKVSCKASGYTFTNYWMHWVRQAPGQGLEWMGRIDPDSTGSKYNEKFKTRVTMTRDTSTSTVYMELSSLRSEDTAVYYCAREGAYGYYFDYWGQGTLVTVSSASTKGPSVFPLAPCSRSTSESTAALGCLVKDYFPEPVTVSWNSGALTSGVHTFPAVLQSSGLYSLSSVVTVPSSSLGTKTYTCNVDHKPSNTKVDKRVESKYGPPCPPCPAPEFLGGPSVFLFPPKPKDTLMISRTPEVTCVVVDVSQEDPEVQFNWYVDGVEVHNAKTKPREEQFNSTYRVVSVLTVLHQDWLNGKEYKCKVSNKGLPSSIEKTISKAKGQPREPQVYTLPPSQEEMTKNQVSLTCLVKGFYPSDIAVEWESNGQPENNYKTTPPVLDSDGSFFLYSRLTVDKSRWQEGNVFSCSVMHEALHNHYTQKSLSLSLGK

SEQ ID NO: 105 - protein, 583 aa, Artificial sequence
  1708-151-21511708C
EVQLVQSGAEVKKPGASVKVSCKASGYTFTNYWMHWVRQAPGQGLEWMGRIDPDSTGSKYNEKFKTRVTMTRDTSTSTVYMELSSLRSEDTAVYYCAREGAYGYYFDYWGQGTLVTVSSASTKGPSVFPLAPCSRSTSESTAALGCLVKDYFPEPVTVSWNSGALTSGVHTFPAVLQSSGLYSLSSVVTVPSSSLGTKTYTCNVDHKPSNTKVDKRVESKYGPPCPPCPAPEFLGGPSVFLFPPKPKDTLMISRTPEVTCVVVDVSQEDPEVQFNWYVDGVEVHNAKTKPREEQFNSTYRVVSVLTVLHQDWLNGKEYKCKVSNKGLPSSIEKTISKAKGQPREPQVYTLPPSQEEMTKNQVSLTCLVKGFYPSDIAVEWESNGQPENNYKTTPPVLDSDGSFFLYSRLTVDKSRWQEGNVFSCSVMHEALHNHYTQKSLSLSLGKGGGGSGGGGSHVQLVESGGGSVQAGGSLRLSCVASASGFTYRPYCMAWFRQAPGKEREAVAGIDIFGGTTYADSVKGRFTASRDNAGFSLFLQMNDLKPEDTAMYYCAAGDSPDGRCPPLGQGLNYWGQGTQVTVSS

SEQ ID NO: 106 - protein, 351 aa, Artificial sequence
  1708-151-31511708N
HVQLVESGGGSVQAGGSLRLSCVASASGFTYRPYCMAWFRQAPGKEREAVAGIDIFGGTTYADSVKGRFTASRDNAGFSLFLQMNDLKPEDTAMYYCAAGDSPDGRCPPLGQGLNYWGQGTQVTVSSGGGGSGGGGSDIQMTQSPSSLSASVGDRVTITCRASENIYSYLAWYQQKPGKSPKLLIYNARTLAEGVPSRFSGSGSGTDFTLTISSLQPEDFATYYCQYHSGSPLPFGGGTKVEIKRTVAAPSVFIFPPSDEQLKSGTASVVCLLNNFYPREAKVQWKVDNALQSGNSQESVTEQDSKDSTYSLSSTLTLSKADYEKHKVYACEVTHQGLSSPVTKSFNRGEC

SEQ ID NO: 107 - protein, 351 aa, Artificial sequence
  1708-151-41511708C
DIQMTQSPSSLSASVGDRVTITCRASENIYSYLAWYQQKPGKSPKLLIYNARTLAEGVPSRFSGSGSGTDFTLTISSLQPEDFATYYCQYHSGSPLPFGGGTKVEIKRTVAAPSVFIFPPSDEQLKSGTASVVCLLNNFYPREAKVQWKVDNALQSGNSQESVTEQDSKDSTYSLSSTLTLSKADYEKHKVYACEVTHQGLSSPVTKSFNRGECGGGGSGGGGSHVQLVESGGGSVQAGGSLRLSCVASASGFTYRPYCMAWFRQAPGKEREAVAGIDIFGGTTYADSVKGRFTASRDNAGFSLFLQMNDLKPEDTAMYYCAAGDSPDGRCPPLGQGLNYWGQGTQVTVSS

SEQ ID NO: 108 - protein, 577 aa, Artificial sequence
  1708-20H5
EVQLVESGGGLVQPGGSLRLSCAASGYTSRTDCMGWFRQAPGKEHEGVAHIDSDGIPRYVDSVKGRFTISQDHAKNSLYLQMNSLRAEDTAVYYCVVGFKFDEDYCAPNDWGQGTMVTVSSGGGGSGGGGSEVQLVQSGAEVKKPGASVKVSCKASGYTFTNYWMHWVRQAPGQGLEWMGRIDPDSTGSKYNEKFKTRVTMTRDTSTSTVYMELSSLRSEDTAVYYCAREGAYGYYFDYWGQGTLVTVSSASTKGPSVFPLAPCSRSTSESTAALGCLVKDYFPEPVTVSWNSGALTSGVHTFPAVLQSSGLYSLSSVVTVPSSSLGTKTYTCNVDHKPSNTKVDKRVESKYGPPCPPCPAPEFLGGPSVFLFPPKPKDTLMISRTPEVTCVVVDVSQEDPEVQFNWYVDGVEVHNAKTKPREEQFNSTYRVVSVLTVLHQDWLNGKEYKCKVSNKGLPSSIEKTISKAKGQPREPQVYTLPPSQEEMTKNQVSLTCLVKGFYPSDIAVEWESNGQPENNYKTTPPVLDSDGSFFLYSRLTVDKSRWQEGNVFSCSVMHEALHNHYTQKSLSLSLGK

SEQ ID NO: 109 - protein, 577 aa, Artificial sequence
  1708-30H2
EVQLVESGGGLVQPGGSLRLSCAASGFTFSGDCMGWFRQAPGKGLDEGVATIDNAGRIKYADSVKGRFTISRDNAKNSLYLQMNSLRAEDTAVYYCAAGWTFGGQCSPADWGQGTQVTVSSGGGGSGGGGSEVQLVQSGAEVKKPGASVKVSCKASGYTFTNYWMHWVRQAPGQGLEWMGRIDPDSTGSKYNEKFKTRVTMTRDTSTSTVYMELSSLRSEDTAVYYCAREGAYGYYFDYWGQGTLVTVSSASTKGPSVFPLAPCSRSTSESTAALGCLVKDYFPEPVTVSWNSGALTSGVHTFPAVLQSSGLYSLSSVVTVPSSSLGTKTYTCNVDHKPSNTKVDKRVESKYGPPCPPCPAPEFLGGPSVFLFPPKPKDTLMISRTPEVTCVVVDVSQEDPEVQFNWYVDGVEVHNAKTKPREEQFNSTYRVVSVLTVLHQDWLNGKEYKCKVSNKGLPSSIEKTISKAKGQPREPQVYTLPPSQEEMTKNQVSLTCLVKGFYPSDIAVEWESNGQPENNYKTTPPVLDSDGSFFLYSRLTVDKSRWQEGNVFSCSVMHEALHNHYTQKSLSLSLGK

SEQ ID NO: 110 - protein, 576 aa, Artificial sequence
  1708-39H2
EVQLVESGGGLVQPGGSLRLSCAASGFTSRTDCMGWFRQAPGKGLEGVAHIDSDGIPRYVESVKGRFTISRDNAKNSLYLQMNSLRAEDTAVYYCVVGFKFGDYCAPNDWGQGTMVTVSSGGGGSGGGGSEVQLVQSGAEVKKPGASVKVSCKASGYTFTNYWMHWVRQAPGQGLEWMGRIDPDSTGSKYNEKFKTRVTMTRDTSTSTVYMELSSLRSEDTAVYYCAREGAYGYYFDYWGQGTLVTVSSASTKGPSVFPLAPCSRSTSESTAALGCLVKDYFPEPVTVSWNSGALTSGVHTFPAVLQSSGLYSLSSVVTVPSSSLGTKTYTCNVDHKPSNTKVDKRVESKYGPPCPPCPAPEFLGGPSVFLFPPKPKDTLMISRTPEVTCVVVDVSQEDPEVQFNWYVDGVEVHNAKTKPREEQFNSTYRVVSVLTVLHQDWLNGKEYKCKVSNKGLPSSIEKTISKAKGQPREPQVYTLPPSQEEMTKNQVSLTCLVKGFYPSDIAVEWESNGQPENNYKTTPPVLDSDGSFFLYSRLTVDKSRWQEGNVFSCSVMHEALHNHYTQKSLSLSLGK

SEQ ID NO: 111 - protein, 583 aa, Artificial sequence
  1708-151H7
HVQLVESGGGLVQPGGSLRLSCVASASGFTYRPYCMAWFRQAPGKEREAVAGIDIFGGTTYADSVKGRFTASRDNAGFSLYLQMNSLRAEDTAVYYCAAGDSPDGRCPPLGQGLNYWGQGTMVTVSSGGGGSGGGGSEVQLVQSGAEVKKPGASVKVSCKASGYTFTNYWMHWVRQAPGQGLEWMGRIDPDSTGSKYNEKFKTRVTMTRDTSTSTVYMELSSLRSEDTAVYYCAREGAYGYYFDYWGQGTLVTVSSASTKGPSVFPLAPCSRSTSESTAALGCLVKDYFPEPVTVSWNSGALTSGVHTFPAVLQSSGLYSLSSVVTVPSSSLGTKTYTCNVDHKPSNTKVDKRVESKYGPPCPPCPAPEFLGGPSVFLFPPKPKDTLMISRTPEVTCVVVDVSQEDPEVQFNWYVDGVEVHNAKTKPREEQFNSTYRVVSVLTVLHQDWLNGKEYKCKVSNKGLPSSIEKTISKAKGQPREPQVYTLPPSQEEMTKNQVSLTCLVKGFYPSDIAVEWESNGQPENNYKTTPPVLDSDGSFFLYSRLTVDKSRWQEGNVFSCSVMHEALHNHYTQKSLSLSLGK

SEQ ID NO: 112 - protein, 583 aa, Artificial sequence
  1708-151H8
EVQLVESGGGLVQPGGSLRLSCVASASGFTYRPYCMAWFRQAPGKGLEAVAGIDIFGGTTYADSVKGRFTISRDNAGFSLYLQMNSLRAEDTAVYYCAAGDSPDGRCPPLGQGLNYWGQGTMVTVSSGGGGSGGGGSEVQLVQSGAEVKKPGASVKVSCKASGYTFTNYWMHWVRQAPGQGLEWMGRIDPDSTGSKYNEKFKTRVTMTRDTSTSTVYMELSSLRSEDTAVYYCAREGAYGYYFDYWGQGTLVTVSSASTKGPSVFPLAPCSRSTSESTAALGCLVKDYFPEPVTVSWNSGALTSGVHTFPAVLQSSGLYSLSSVVTVPSSSLGTKTYTCNVDHKPSNTKVDKRVESKYGPPCPPCPAPEFLGGPSVFLFPPKPKDTLMISRTPEVTCVVVDVSQEDPEVQFNWYVDGVEVHNAKTKPREEQFNSTYRVVSVLTVLHQDWLNGKEYKCKVSNKGLPSSIEKTISKAKGQPREPQVYTLPPSQEEMTKNQVSLTCLVKGFYPSDIAVEWESNGQPENNYKTTPPVLDSDGSFFLYSRLTVDKSRWQEGNVFSCSVMHEALHNHYTQKSLSLSLGK

SEQ ID NO: 113 - protein, 449 aa, Artificial sequence
  1708-IgG1 (1708IgG1) HC
EVQLVQSGAEVKKPGASVKVSCKASGYTFTNYWMHWVRQAPGQGLEWMGRIDPDSTGSKYNEKFKTRVTMTRDTSTSTVYMELSSLRSEDTAVYYCAREGAYGYYFDYWGQGTLVTVSSASTKGPSVFPLAPSSKSTSGGTAALGCLVKDYFPEPVTVSWNSGALTSGVHTFPAVLQSSGLYSLSSVVTVPSSSLGTQTYICNVNHKPSNTKVDKKVEPKSCDKTHTCPPCPAPELLGGPSVFLFPPKPKDTLMISRTPEVTCVVVDVSHEDPEVKFNWYVDGVEVHNAKTKPREEQYNSTYRVVSVLTVLHQDWLNGKEYKCKVSNKALPAPIEKTISKAKGQPREPQVYTLPPSREEMTKNQVSLTCLVKGFYPSDIAVEWESNGQPENNYKTTPPVLDSDGSFFLYSKLTVDKSRWQQGNVFSCSVMHEALHNHYTQKSLSLSPGK

SEQ ID NO: 114 - protein, 586 aa, Artificial sequence
  1708-151-IgG1 (1708-151IgG1)
HVQLVESGGGSVQAGGSLRLSCVASASGFTYRPYCMAWFRQAPGKEREAVAGIDIFGGTTYADSVKGRFTASRDNAGFSLFLQMNDLKPEDTAMYYCAAGDSPDGRCPPLGQGLNYWGQGTQVTVSSGGGGSGGGGSEVQLVQSGAEVKKPGASVKVSCKASGYTFTNYWMHWVRQAPGQGLEWMGRIDPDSTGSKYNEKFKTRVTMTRDTSTSTVYMELSSLRSEDTAVYYCAREGAYGYYFDYWGQGTLVTVSSASTKGPSVFPLAPSSKSTSGGTAALGCLVKDYFPEPVTVSWNSGALTSGVHTFPAVLQSSGLYSLSSVVTVPSSSLGTQTYICNVNHKPSNTKVDKKVEPKSCDKTHTCPPCPAPELLGGPSVFLFPPKPKDTLMISRTPEVTCVVVDVSHEDPEVKFNWYVDGVEVHNAKTKPREEQYNSTYRVVSVLTVLHQDWLNGKEYKCKVSNKALPAPIEKTISKAKGQPREPQVYTLPPSREEMTKNQVSLTCLVKGFYPSDIAVEWESNGQPENNYKTTPPVLDSDGSFFLYSKLTVDKSRWQQGNVFSCSVMHEALHNHYTQKSLSLSPGK

SEQ ID NO: 115 - protein, 5 aa, Artificial sequence
  1707 HCDR1
DYHMY

SEQ ID NO: 116 - protein, 17 aa, Artificial sequence
  1707 HCDR2
YISKGGISTYYPDTVKG

SEQ ID NO: 117 - protein, 10 aa, Artificial sequence
  1707 HCDR3
QSSYDFAMDY

SEQ ID NO: 118 - protein, 11 aa, Artificial sequence
  1707 LCDR1
KASQDVGTSVA

SEQ ID NO: 119 - protein, 7 aa, Artificial sequence
  1707 LCDR2
WASARHT

SEQ ID NO: 120 - protein, 9 aa, Artificial sequence
  1707 LCDR3
QQYSSYPLT

SEQ ID NO: 121 - protein, 5 aa, Artificial sequence
  1708 HCDR1
NYWMH

SEQ ID NO: 122 - protein, 17 aa, Artificial sequence
  1708 HCDR2
RIDPDSTGSKYNEKFKT

SEQ ID NO: 123 - protein, 10 aa, Artificial sequence
  1708 HCDR3
EGAYGYYFDY

SEQ ID NO: 124 - protein, 11 aa, Artificial sequence
  1708 LCDR1
RASENIYSYLA

SEQ ID NO: 125 - protein, 7 aa, Artificial sequence
  1708 LCDR2
NARTLAE

SEQ ID NO: 126 - protein, 9 aa, Artificial sequence
  1708 LCDR3
QYHSGSPLP

SEQ ID NO: 127 - protein, 5 aa, Artificial sequence
  1709 HCDR1
DYYMH

SEQ ID NO: 128 - protein, 17 aa, Artificial sequence
  1709 HCDR2
LVYPYNDNTGYNRKFKG

SEQ ID NO: 129 - protein, 11 aa, Artificial sequence
  1709 HCDR3
GGPSNWNYFDY

SEQ ID NO: 130 - protein, 11 aa, Artificial sequence
  1709 LCDR1
KASQNVVTAVA

SEQ ID NO: 131 - protein, 7 aa, Artificial sequence
  1709 LCDR2
SASNRYT

SEQ ID NO: 132 - protein, 9 aa, Artificial sequence
  1709 HCDR3
QQYTLYPLT

SEQ ID NO: 133 - protein, 5 aa, Artificial sequence
  1710 HCDR1
NYYMH

SEQ ID NO: 134 - protein, 17 aa, Artificial sequence
  1710 HCDR2
RIDPTSGATKYNDNFKG

SEQ ID NO: 135 - protein, 10 aa, Artificial sequence
  1710 HCDR3
EGGFGYYFDY

SEQ ID NO: 136 - protein, 11 aa, Artificial sequence
  1710 LCDR1
RTSENIFTYLA

SEQ ID NO: 137 - protein, 7 aa, Artificial sequence
  1710 LCDR2
NAKTFAE

SEQ ID NO: 138 - protein, 9 aa, Artificial sequence
  1710 LCDR3
QHHYGIPLP

SEQ ID NO: 139 - protein, 5 aa, Artificial sequence
  1711 HCDR1
NYWIG

SEQ ID NO: 140 - protein, 17 aa, Artificial sequence
  1711 HCDR2
DIYPGGAYTNYNEKFKD

SEQ ID NO: 141 - protein, 13 aa, Artificial sequence
  1711 HCDR3
GDYYDSSGRAMDY

SEQ ID NO: 142 - protein, 17 aa, Artificial sequence
  1711 LCDR1
KSSQSLLYSRNQMNYLA

SEQ ID NO: 143 - protein, 7 aa, Artificial sequence
  1711 LCDR2
WTSTRES

SEQ ID NO: 144 - protein, 9 aa, Artificial sequence
  1711 LCDR3
QQYYSYPYT

SEQ ID NO: 145 - protein, 119 aa, Artificial sequence
  1708-VH1
EVQLVQSGAEVKKPGASVKVSCKASGYTFTNYWMHWVRQAPGQGLEWMGRIDPDSTGSKYNEKFKTRVTMTRDTSTSTVYMELSSLRSEDTAVYYCAREGAYGYYFDYWGQGTLVTVSS

SEQ ID NO: 146 - protein, 119 aa, Artificial sequence
  1708-VH2
EVQLVQSGAEVKKPGASVKVSCKASGYTFTNYWMHWVRQAPGQGLEWMGRIDPDSTGSKYNEKFKTRVTMTVDTSTSTVYMELSSLRSEDTAVYYCAREGAYGYYFDYWGQGTLVTVSS

SEQ ID NO: 147 - protein, 119 aa, Artificial sequence
  1708-VH3
EVQLVQSGAEVKKPGASVKVSCKASGYTFTNYWMHWVRQAPGQGLEWIGRIDPDSTGSKYNEKFKTRVTMTVDTSTSTAYMELSSLRSEDTAVYYCAREGAYGYYFDYWGQGTLVTVSS

SEQ ID NO: 148 - protein, 107 aa, Artificial sequence
  1708-VL1
DIQMTQSPSSLSASVGDRVTITCRASENIYSYLAWYQQKPGKAPKLLIYNARTLAEGVPSRFSGSGSGTDFTLTISSLQPEDFATYYCQYHSGSPLPFGGGTKVEIK

SEQ ID NO: 149 - protein, 107 aa, Artificial sequence
  1708-VL2
DIQMTQSPSSLSASVGDRVTITCRASENIYSYLAWYQQKPGKSPKLLIYNARTLAEGVPSRFSGSGSGTDFTLTISSLQPEDFATYYCQYHSGSPLPFGGGTKVEIK

SEQ ID NO: 150 - protein, 13 aa, Artificial sequence
  20 HCDR3
GFKFDEDYCAPND

SEQ ID NO: 151 - protein, 12 aa, Artificial sequence
  30 HCDR3
GWTFGGQCSPAD

SEQ ID NO: 152 - protein, 10 aa, Artificial sequence
  Linker
GGGGSGGGGS

SEQ ID NO: 153 - protein, 229 aa, Artificial sequence
  Fc region of human IgG4 heavy chain (S228P/K447A)
ESKYGPPCPPCPAPEFLGGPSVFLFPPKPKDTLMISRTPEVTCVVVDVSQEDPEVQFNWYVDGVEVHNAKTKPREEQFNSTYRVVSVLTVLHQDWLNGKEYKCKVSNKGLPSSIEKTISKAKGQPREPQVYTLPPSQEEMTKNQVSLTCLVKGFYPSDIAVEWESNGQPENNYKTTPPVLDSDGSFFLYSRLTVDKSRWQEGNVFSCSVMHEALHNHYTQKSLSLSLGK